European Patent Application EP 4 628 581 A1, published October 8, 2025. Title: Novel Fumonisin degrading enzyme and use thereof. Applicant: CJ CheilJedang Corporation. Application KR. The sequence listing filed with the application follows.

SEQUENCE LISTING (4 sequences)

SEQ ID NO: 1 - protein, 488 aa, synthetic construct
  source 1..488: note = EFB1-9
MEPVIVQTSTGALAGSGGDIRVFKGVPFGAPPIGALRWRPPEPPTPWQGVRDATQFGADCMQKRLPDTRAPGVSEDCLTLNIWAPAQNSGGALPVMVWVYGGGFVDGSASLPIYDGEALARKGVVVVTVNYRTGVFGFLAHPALAAESPHHSAGNYGILDVIAALRWLKSNVAAFGGDPNRVTVFGESAGASLLDMVLVSPLSEGLVHGAILESPGAMRPLSSLTDASEIGKIVGPDIAAMREMSAEQVLAMTDRIVPAVRRLTTPRALGPILDGWVVPRTDTAAFATGEIHRVPLIVGGNSDEGRLFVRNWPIHTVDEARAYADTNFGASAGELMALYKFDKDAAVPSALSYAFGDTQFNYGVRGLARGMSKVQPKTFRYLFTRSPGGVPPAPTHSEEIDYALANLGAHRFIPRGAFDATDRTLSAAMADAWVRFASTGDPNGGMLPHWPAYDGESDPYLEFGDSIRVGQGYRTTYLDFVESFLTKP

SEQ ID NO: 2 - DNA, 1464 bp, synthetic construct
  source 1..1464: mol_type = other DNA; note = EFB1-9
atggagcccgtcatcgttcaaacttcaactggagctcttgcgggcagcggcggggatataagagtattcaaaggggtgccattcggtgcgcctccgattggagcattaagatggagaccacctgaaccccccacgccttggcagggtgtacgtgacgctacgcagttcggggctgactgtatgcagaaaagactgccagacacgcgcgcaccgggcgtatcagaggactgcttgacattaaatatctgggcaccagcccagaatagtggcggcgcactgcccgttatggtctgggtctatgggggcggatttgtcgacggttcagcatctcttcccatctacgacggggaggcattagctcgcaaaggcgttgtcgttgttacggttaactatagaacaggtgtgttcgggtttttagctcatcccgccttagcggcggagagtccgcatcatagtgcggggaactacggtatcttagacgtgattgccgcgctgagatggttaaaatcgaacgtggcggccttcggaggggaccctaatcgggtcacggtatttggagaaagtgcaggagcttcattgttggatatggtgttggtttcgccgctgagtgaaggcttggtacatggcgccatactggaatctccgggggcaatgcgtccactttcgtcattaaccgacgcgtccgaaatcggtaaaatagtggggccagatatagcggccatgcgtgaaatgtcggcggaacaagtacttgctatgactgatcgtattgtcccggctgtccgccgtctgacgacaccccgtgcgttaggcccaatcttggacggttgggtagtaccacggacagacacggcggcgtttgcgactggcgagatacacagagtaccgcttattgttggcggaaattcagatgaagggcggctgttcgttcggaattggccaatccatactgttgatgaagcacgcgcgtatgcggacacgaatttcggagcgagtgcgggagagctgatggccttatacaaattcgacaaagacgccgcagtgccatccgcgttaagttacgcattcggggacacgcaatttaattatggtgtccgtgggctggcacgcggcatgtccaaggtgcagccaaaaacgtttcgctatttgtttacccgttcgccaggcggggttcccccagcgcccacgcactccgaggaaatcgactatgccttagccaacctgggcgctcatcggtttatccctcggggcgccttcgatgcaaccgaccgcaccttaagtgcagcgatggcggacgcgtgggtccggtttgcctccactggagaccctaatgggggcatgttgcctcattggcctgcgtatgatggcgaatcggatccctaccttgagttcggcgattctataagagtaggccaaggctatagaacaacgtacttagacttcgtcgagagtttcttaaccaaaccg

SEQ ID NO: 3 - DNA, 36 bp, synthetic construct
  source 1..36: mol_type = other DNA
cggcagccatatggagcccgtcatcgttcaaacttc

SEQ ID NO: 4 - DNA, 39 bp, synthetic construct
  source 1..39: mol_type = other DNA
tcgagtgcggccgctcacggtttggttaagaaactctcg